European Patent Specification EP 4 008 796 B1, published August 9, 2023. Title: Construction of Next Generation Sequencing (NGS) Libraries Using Competitive Strand Displacement. Applicant: Integrated DNA Technologies, Inc. Application EP. The sequence listing filed with the application follows.

SEQUENCE LISTING (98 sequences)

SEQ ID NO: 1 - DNA, 58 bp, Artificial Sequence
  Synthetic
aatgatacggcgaccaccgagatctacactctttccctacacgacgctcttccgatct

SEQ ID NO: 2 - DNA, 68 bp, Artificial Sequence
  synthetic nucleic acid
  misc_feature (30)..(35): UMI
aatgatacggcgaccaccgagatctacacnnnnnnacactctttccctacacgacgctcttccgatct

SEQ ID NO: 3 - DNA, 70 bp, Artificial Sequence
  synthetic nucleic acid
  misc_feature (1)..(1): 5Phos
  misc_feature (35)..(40): UMI
agatcggaagagcacacgtctgaactccagtcacnnnnnnatcacgatctcgtatgccgtcttctgcttg

SEQ ID NO: 4 - DNA, 70 bp, Artificial Sequence
  synthetic nucleic acid
  misc_feature (1)..(1): 5Phos
  misc_feature (35)..(40): UMI
agatcggaagagcacacgtctgaactccagtcacnnnnnncgatgtatctcgtatgccgtcttctgcttg

SEQ ID NO: 5 - DNA, 70 bp, Artificial Sequence
  synthetic nucleic acid
  misc_feature (1)..(1): 5Phos
  misc_feature (35)..(40): UMI
agatcggaagagcacacgtctgaactccagtcacnnnnnnttaggcatctcgtatgccgtcttctgcttg

SEQ ID NO: 6 - DNA, 70 bp, Artificial Sequence
  synthetic nucleic acid
  misc_feature (1)..(1): 5Phos
  misc_feature (35)..(40): UMI
agatcggaagagcacacgtctgaactccagtcacnnnnnntgaccaatctcgtatgccgtcttctgcttg

SEQ ID NO: 7 - DNA, 70 bp, Artificial Sequence
  synthetic nucleic acid
  misc_feature (1)..(1): 5Phos
  misc_feature (35)..(40): UMI
agatcggaagagcacacgtctgaactccagtcacnnnnnnacagtgatctcgtatgccgtcttctgcttg

SEQ ID NO: 8 - DNA, 70 bp, Artificial Sequence
  synthetic nucleic acid
  misc_feature (1)..(1): 5Phos
  misc_feature (35)..(40): UMI
agatcggaagagcacacgtctgaactccagtcacnnnnnngccaatatctcgtatgccgtcttctgcttg

SEQ ID NO: 9 - DNA, 70 bp, Artificial Sequence
  synthetic nucleic acid
  misc_feature (1)..(1): 5Phos
  misc_feature (35)..(40): UMI
agatcggaagagcacacgtctgaactccagtcacnnnnnncagatcatctcgtatgccgtcttctgcttg

SEQ ID NO: 10 - DNA, 70 bp, Artificial Sequence
  synthetic nucleic acid
  misc_feature (1)..(1): 5Phos
  misc_feature (35)..(40): UMI
agatcggaagagcacacgtctgaactccagtcacnnnnnnacttgaatctcgtatgccgtcttctgcttg

SEQ ID NO: 11 - DNA, 72 bp, Artificial Sequence
  synthetic nucleic acid
  misc_feature (1)..(1): 5rApp
  misc_feature (43)..(48): UMI
  misc_feature (72)..(72): 3SpC3
agatcggaagagcacacgtctgaactccagtcacaacggcggnnnnnnatctcgtatgccgtcttctgcttg

SEQ ID NO: 12 - DNA, 72 bp, Artificial Sequence
  synthetic nucleic acid
  misc_feature (1)..(1): 5rApp
  misc_feature (43)..(48): UMI
  misc_feature (72)..(72): 3SpC3
agatcggaagagcacacgtctgaactccagtcaccatccgttnnnnnnatctcgtatgccgtcttctgcttg

SEQ ID NO: 13 - DNA, 72 bp, Artificial Sequence
  synthetic nucleic acid
  misc_feature (1)..(1): 5rApp
  misc_feature (43)..(48): UMI
  misc_feature (72)..(72): 3SpC3
agatcggaagagcacacgtctgaactccagtcaccgaattggnnnnnnatctcgtatgccgtcttctgcttg

SEQ ID NO: 14 - DNA, 72 bp, Artificial Sequence
  synthetic nucleic acid
  misc_feature (1)..(1): 5rApp
  misc_feature (43)..(48): UMI
  misc_feature (72)..(72): 3SpC3
agatcggaagagcacacgtctgaactccagtcacttagaaccnnnnnnatctcgtatgccgtcttctgcttg

SEQ ID NO: 15 - DNA, 72 bp, Artificial Sequence
  synthetic nucleic acid
  misc_feature (1)..(1): 5rApp
  misc_feature (43)..(48): UMI
  misc_feature (72)..(72): 3SpC3
agatcggaagagcacacgtctgaactccagtcacggccaacgnnnnnnatctcgtatgccgtcttctgcttg

SEQ ID NO: 16 - DNA, 72 bp, Artificial Sequence
  synthetic nucleic acid
  misc_feature (1)..(1): 5rApp
  misc_feature (43)..(48): UMI
  misc_feature (72)..(72): 3SpC3
agatcggaagagcacacgtctgaactccagtcactcttggttnnnnnnatctcgtatgccgtcttctgcttg

SEQ ID NO: 17 - DNA, 12 bp, Artificial Sequence
  synthetic nucleic acid
  misc_feature (12)..(12): ddT
ctcttccgatct

SEQ ID NO: 18 - DNA, 42 bp, Artificial Sequence
  synthetic nucleic acid
  misc_feature (1)..(1): 5rApp
  misc_feature (1)..(8): UMI
  misc_feature (42)..(42): 3SpC3
acgatcagagatcggaagagcacacgtctgaactccagtcac

SEQ ID NO: 19 - DNA, 42 bp, Artificial Sequence
  synthetic nucleic acid
  misc_feature (1)..(1): 5rApp
  misc_feature (1)..(8): UMI
  misc_feature (42)..(42): 3SpC3
tcgagagtagatcggaagagcacacgtctgaactccagtcac

SEQ ID NO: 20 - DNA, 42 bp, Artificial Sequence
  synthetic nucleic acid
  misc_feature (1)..(1): 5rApp
  misc_feature (1)..(8): UMI
  misc_feature (42)..(42): 3SpC3
ctagctcaagatcggaagagcacacgtctgaactccagtcac

SEQ ID NO: 21 - DNA, 42 bp, Artificial Sequence
  synthetic nucleic acid
  misc_feature (1)..(1): 5rApp
  misc_feature (1)..(8): UMI
  misc_feature (42)..(42): 3SpC3
atcgtctcagatcggaagagcacacgtctgaactccagtcac

SEQ ID NO: 22 - DNA, 42 bp, Artificial Sequence
  synthetic nucleic acid
  misc_feature (1)..(1): 5rApp
  misc_feature (1)..(8): UMI
  misc_feature (42)..(42): 3SpC3
tcgacaagagatcggaagagcacacgtctgaactccagtcac

SEQ ID NO: 23 - DNA, 42 bp, Artificial Sequence
  synthetic nucleic acid
  misc_feature (1)..(1): 5rApp
  misc_feature (1)..(8): UMI
  misc_feature (42)..(42): 3SpC3
ccttggaaagatcggaagagcacacgtctgaactccagtcac

SEQ ID NO: 24 - DNA, 42 bp, Artificial Sequence
  synthetic nucleic acid
  misc_feature (1)..(1): 5rApp
  misc_feature (1)..(8): UMI
  misc_feature (42)..(42): 3SpC3
atcatgcgagatcggaagagcacacgtctgaactccagtcac

SEQ ID NO: 25 - DNA, 42 bp, Artificial Sequence
  synthetic nucleic acid
  misc_feature (1)..(1): 5rApp
  misc_feature (1)..(8): UMI
  misc_feature (42)..(42): 3SpC3
tgttccgtagatcggaagagcacacgtctgaactccagtcac

SEQ ID NO: 26 - DNA, 42 bp, Artificial Sequence
  synthetic nucleic acid
  misc_feature (1)..(1): 5rApp
  misc_feature (1)..(8): UMI
  misc_feature (42)..(42): 3SpC3
attagccgagatcggaagagcacacgtctgaactccagtcac

SEQ ID NO: 27 - DNA, 42 bp, Artificial Sequence
  synthetic nucleic acid
  misc_feature (1)..(1): 5rApp
  misc_feature (1)..(8): UMI
  misc_feature (42)..(42): 3SpC3
cgatcgatagatcggaagagcacacgtctgaactccagtcac

SEQ ID NO: 28 - DNA, 42 bp, Artificial Sequence
  synthetic nucleic acid
  misc_feature (1)..(1): 5rApp
  misc_feature (1)..(8): UMI
  misc_feature (42)..(42): 3SpC3
gatcttgcagatcggaagagcacacgtctgaactccagtcac

SEQ ID NO: 29 - DNA, 42 bp, Artificial Sequence
  synthetic nucleic acid
  misc_feature (1)..(1): 5rApp
  misc_feature (1)..(8): UMI
  misc_feature (42)..(42): 3SpC3
aggatagcagatcggaagagcacacgtctgaactccagtcac

SEQ ID NO: 30 - DNA, 42 bp, Artificial Sequence
  synthetic nucleic acid
  misc_feature (1)..(1): 5rApp
  misc_feature (1)..(8): UMI
  misc_feature (42)..(42): 3SpC3
gtagcgtaagatcggaagagcacacgtctgaactccagtcac

SEQ ID NO: 31 - DNA, 42 bp, Artificial Sequence
  synthetic nucleic acid
  misc_feature (1)..(1): 5rApp
  misc_feature (1)..(8): UMI
  misc_feature (42)..(42): 3SpC3
agagtccaagatcggaagagcacacgtctgaactccagtcac

SEQ ID NO: 32 - DNA, 42 bp, Artificial Sequence
  synthetic nucleic acid
  misc_feature (1)..(1): 5rApp
  misc_feature (1)..(8): UMI
  misc_feature (42)..(42): 3SpC3
gctactctagatcggaagagcacacgtctgaactccagtcac

SEQ ID NO: 33 - DNA, 42 bp, Artificial Sequence
  synthetic nucleic acid
  misc_feature (1)..(1): 5rApp
  misc_feature (1)..(8): UMI
  misc_feature (42)..(42): 3SpC3
ctctggatagatcggaagagcacacgtctgaactccagtcac

SEQ ID NO: 34 - DNA, 10 bp, Artificial Sequence
  synthetic nucleic acid
  misc_feature (3)..(9): UMI
  misc_feature (10)..(10): ddT
ctctgatcgt

SEQ ID NO: 35 - DNA, 10 bp, Artificial Sequence
  synthetic nucleic acid
  misc_feature (3)..(9): UMI
  misc_feature (10)..(10): ddA
ctactctcga

SEQ ID NO: 36 - DNA, 10 bp, Artificial Sequence
  synthetic nucleic acid
  misc_feature (3)..(9): UMI
  misc_feature (10)..(10): ddG
cttgagctag

SEQ ID NO: 37 - DNA, 10 bp, Artificial Sequence
  synthetic nucleic acid
  misc_feature (3)..(9): UMI
  misc_feature (10)..(10): ddT
ctgagacgat

SEQ ID NO: 38 - DNA, 10 bp, Artificial Sequence
  synthetic nucleic acid
  misc_feature (3)..(9): UMI
  misc_feature (10)..(10): ddA
ctcttgtcga

SEQ ID NO: 39 - DNA, 10 bp, Artificial Sequence
  synthetic nucleic acid
  misc_feature (3)..(9): UMI
  misc_feature (10)..(10): ddG
ctttccaagg

SEQ ID NO: 40 - DNA, 10 bp, Artificial Sequence
  synthetic nucleic acid
  misc_feature (3)..(9): UMI
  misc_feature (10)..(10): ddT
ctcgcatgat

SEQ ID NO: 41 - DNA, 10 bp, Artificial Sequence
  synthetic nucleic acid
  misc_feature (3)..(9): UMI
  misc_feature (10)..(10): ddA
ctacggaaca

SEQ ID NO: 42 - DNA, 10 bp, Artificial Sequence
  synthetic nucleic acid
  misc_feature (3)..(9): UMI
  misc_feature (10)..(10): ddT
ctcggctaat

SEQ ID NO: 43 - DNA, 10 bp, Artificial Sequence
  synthetic nucleic acid
  misc_feature (3)..(9): UMI
  misc_feature (10)..(10): ddG
ctatcgatcg

SEQ ID NO: 44 - DNA, 10 bp, Artificial Sequence
  synthetic nucleic acid
  misc_feature (3)..(9): UMI
  misc_feature (10)..(10): ddC
ctgcaagatc

SEQ ID NO: 45 - DNA, 10 bp, Artificial Sequence
  synthetic nucleic acid
  misc_feature (3)..(9): UMI
  misc_feature (10)..(10): ddT
ctgctatcct

SEQ ID NO: 46 - DNA, 10 bp, Artificial Sequence
  synthetic nucleic acid
  misc_feature (3)..(9): UMI
  misc_feature (10)..(10): ddC
cttacgctac

SEQ ID NO: 47 - DNA, 10 bp, Artificial Sequence
  synthetic nucleic acid
  misc_feature (3)..(9): UMI
  misc_feature (10)..(10): ddT
cttggactct

SEQ ID NO: 48 - DNA, 10 bp, Artificial Sequence
  synthetic nucleic acid
  misc_feature (3)..(9): UMI
  misc_feature (10)..(10): ddC
ctagagtagc

SEQ ID NO: 49 - DNA, 10 bp, Artificial Sequence
  synthetic nucleic acid
  misc_feature (3)..(9): UMI
  misc_feature (10)..(10): ddG
ctatccagag

SEQ ID NO: 50 - DNA, 33 bp, Artificial Sequence
  synthetic nucleic acid
acactctttccctacacgacgctcttccgatct

SEQ ID NO: 51 - DNA, 53 bp, Artificial Sequence
  synthetic nucleic acid
  misc_feature (25)..(32): sample barcode
caagcagaagacggcatacgagatctgatcgtgtgactggagttcagacgtgt

SEQ ID NO: 52 - DNA, 53 bp, Artificial Sequence
  synthetic nucleic acid
  misc_feature (25)..(32): sample barcode
caagcagaagacggcatacgagatactctcgagtgactggagttcagacgtgt

SEQ ID NO: 53 - DNA, 53 bp, Artificial Sequence
  synthetic nucleic acid
  misc_feature (25)..(32): sample barcode
caagcagaagacggcatacgagattgagctaggtgactggagttcagacgtgt

SEQ ID NO: 54 - DNA, 53 bp, Artificial Sequence
  synthetic nucleic acid
  misc_feature (25)..(32): sample barcode
caagcagaagacggcatacgagatgagacgatgtgactggagttcagacgtgt

SEQ ID NO: 55 - DNA, 53 bp, Artificial Sequence
  synthetic nucleic acid
  misc_feature (25)..(32): sample barcode
caagcagaagacggcatacgagatcttgtcgagtgactggagttcagacgtgt

SEQ ID NO: 56 - DNA, 53 bp, Artificial Sequence
  synthetic nucleic acid
  misc_feature (25)..(32): sample barcode
caagcagaagacggcatacgagatttccaagggtgactggagttcagacgtgt

SEQ ID NO: 57 - DNA, 53 bp, Artificial Sequence
  synthetic nucleic acid
  misc_feature (25)..(32): sample barcode
caagcagaagacggcatacgagatcgcatgatgtgactggagttcagacgtgt

SEQ ID NO: 58 - DNA, 53 bp, Artificial Sequence
  synthetic nucleic acid
  misc_feature (25)..(32): sample barcode
caagcagaagacggcatacgagatacggaacagtgactggagttcagacgtgt

SEQ ID NO: 59 - DNA, 53 bp, Artificial Sequence
  synthetic nucleic acid
  misc_feature (25)..(32): sample barcode
caagcagaagacggcatacgagatcggctaatgtgactggagttcagacgtgt

SEQ ID NO: 60 - DNA, 53 bp, Artificial Sequence
  synthetic nucleic acid
  misc_feature (25)..(32): sample barcode
caagcagaagacggcatacgagatatcgatcggtgactggagttcagacgtgt

SEQ ID NO: 61 - DNA, 53 bp, Artificial Sequence
  synthetic nucleic acid
  misc_feature (25)..(32): sample barcode
caagcagaagacggcatacgagatgcaagatcgtgactggagttcagacgtgt

SEQ ID NO: 62 - DNA, 53 bp, Artificial Sequence
  synthetic nucleic acid
  misc_feature (25)..(32): sample barcode
caagcagaagacggcatacgagatgctatcctgtgactggagttcagacgtgt

SEQ ID NO: 63 - DNA, 53 bp, Artificial Sequence
  synthetic nucleic acid
  misc_feature (25)..(32): sample barcode
caagcagaagacggcatacgagattacgctacgtgactggagttcagacgtgt

SEQ ID NO: 64 - DNA, 53 bp, Artificial Sequence
  synthetic nucleic acid
  misc_feature (25)..(32): sample barcode
caagcagaagacggcatacgagattggactctgtgactggagttcagacgtgt

SEQ ID NO: 65 - DNA, 53 bp, Artificial Sequence
  synthetic nucleic acid
  misc_feature (25)..(32): sample barcode
caagcagaagacggcatacgagatagagtagcgtgactggagttcagacgtgt

SEQ ID NO: 66 - DNA, 53 bp, Artificial Sequence
  synthetic nucleic acid
  misc_feature (25)..(32): sample barcode
caagcagaagacggcatacgagatatccagaggtgactggagttcagacgtgt

SEQ ID NO: 67 - DNA, 53 bp, Artificial Sequence
  synthetic nucleic acid
  misc_feature (25)..(32): sample barcode
caagcagaagacggcatacgagatgacgatctgtgactggagttcagacgtgt

SEQ ID NO: 68 - DNA, 53 bp, Artificial Sequence
  synthetic nucleic acid
  misc_feature (25)..(32): sample barcode
caagcagaagacggcatacgagataactgagcgtgactggagttcagacgtgt

SEQ ID NO: 69 - DNA, 53 bp, Artificial Sequence
  synthetic nucleic acid
  misc_feature (25)..(32): sample barcode
caagcagaagacggcatacgagatcttaggacgtgactggagttcagacgtgt

SEQ ID NO: 70 - DNA, 53 bp, Artificial Sequence
  synthetic nucleic acid
  misc_feature (25)..(32): sample barcode
caagcagaagacggcatacgagatgtgccatagtgactggagttcagacgtgt

SEQ ID NO: 71 - DNA, 53 bp, Artificial Sequence
  synthetic nucleic acid
  misc_feature (25)..(32): sample barcode
caagcagaagacggcatacgagatgaatccgagtgactggagttcagacgtgt

SEQ ID NO: 72 - DNA, 53 bp, Artificial Sequence
  synthetic nucleic acid
  misc_feature (25)..(32): sample barcode
caagcagaagacggcatacgagattcgctgttgtgactggagttcagacgtgt

SEQ ID NO: 73 - DNA, 53 bp, Artificial Sequence
  synthetic nucleic acid
  misc_feature (25)..(32): sample barcode
caagcagaagacggcatacgagatttcgttgggtgactggagttcagacgtgt

SEQ ID NO: 74 - DNA, 53 bp, Artificial Sequence
  synthetic nucleic acid
  misc_feature (25)..(32): sample barcode
caagcagaagacggcatacgagataagcactggtgactggagttcagacgtgt

SEQ ID NO: 75 - DNA, 57 bp, Artificial Sequence
  synthetic nucleic acid
  misc_feature (30)..(37): sample barcode
aatgatacggcgaccaccgagatctacacctgatcgtacactctttccctacacgac

SEQ ID NO: 76 - DNA, 57 bp, Artificial Sequence
  synthetic nucleic acid
  misc_feature (30)..(37): sample barcode
aatgatacggcgaccaccgagatctacacactctcgaacactctttccctacacgac

SEQ ID NO: 77 - DNA, 57 bp, Artificial Sequence
  synthetic nucleic acid
  misc_feature (30)..(37): sample barcode
aatgatacggcgaccaccgagatctacactgagctagacactctttccctacacgac

SEQ ID NO: 78 - DNA, 57 bp, Artificial Sequence
  synthetic nucleic acid
  misc_feature (30)..(37): sample barcode
aatgatacggcgaccaccgagatctacacgagacgatacactctttccctacacgac

SEQ ID NO: 79 - DNA, 57 bp, Artificial Sequence
  synthetic nucleic acid
  misc_feature (30)..(37): sample barcode
aatgatacggcgaccaccgagatctacaccttgtcgaacactctttccctacacgac

SEQ ID NO: 80 - DNA, 57 bp, Artificial Sequence
  synthetic nucleic acid
  misc_feature (30)..(37): sample barcode
aatgatacggcgaccaccgagatctacacttccaaggacactctttccctacacgac

SEQ ID NO: 81 - DNA, 57 bp, Artificial Sequence
  synthetic nucleic acid
  misc_feature (30)..(37): sample barcode
aatgatacggcgaccaccgagatctacaccgcatgatacactctttccctacacgac

SEQ ID NO: 82 - DNA, 57 bp, Artificial Sequence
  synthetic nucleic acid
  misc_feature (30)..(37): sample barcode
aatgatacggcgaccaccgagatctacacacggaacaacactctttccctacacgac

SEQ ID NO: 83 - DNA, 57 bp, Artificial Sequence
  synthetic nucleic acid
  misc_feature (30)..(37): sample barcode
aatgatacggcgaccaccgagatctacaccggctaatacactctttccctacacgac

SEQ ID NO: 84 - DNA, 57 bp, Artificial Sequence
  synthetic nucleic acid
  misc_feature (30)..(37): sample barcode
aatgatacggcgaccaccgagatctacacatcgatcgacactctttccctacacgac

SEQ ID NO: 85 - DNA, 57 bp, Artificial Sequence
  synthetic nucleic acid
  misc_feature (30)..(37): sample barcode
aatgatacggcgaccaccgagatctacacgcaagatcacactctttccctacacgac

SEQ ID NO: 86 - DNA, 57 bp, Artificial Sequence
  synthetic nucleic acid
  misc_feature (30)..(37): sample barcode
aatgatacggcgaccaccgagatctacacgctatcctacactctttccctacacgac

SEQ ID NO: 87 - DNA, 57 bp, Artificial Sequence
  synthetic nucleic acid
  misc_feature (30)..(37): sample barcode
aatgatacggcgaccaccgagatctacactacgctacacactctttccctacacgac

SEQ ID NO: 88 - DNA, 57 bp, Artificial Sequence
  synthetic nucleic acid
  misc_feature (30)..(37): sample barcode
aatgatacggcgaccaccgagatctacactggactctacactctttccctacacgac

SEQ ID NO: 89 - DNA, 57 bp, Artificial Sequence
  synthetic nucleic acid
  misc_feature (30)..(37): sample barcode
aatgatacggcgaccaccgagatctacacagagtagcacactctttccctacacgac

SEQ ID NO: 90 - DNA, 57 bp, Artificial Sequence
  synthetic nucleic acid
  misc_feature (30)..(37): sample barcode
aatgatacggcgaccaccgagatctacacatccagagacactctttccctacacgac

SEQ ID NO: 91 - DNA, 57 bp, Artificial Sequence
  synthetic nucleic acid
  misc_feature (30)..(37): sample barcode
aatgatacggcgaccaccgagatctacacgacgatctacactctttccctacacgac

SEQ ID NO: 92 - DNA, 57 bp, Artificial Sequence
  synthetic nucleic acid
  misc_feature (30)..(37): sample barcode
aatgatacggcgaccaccgagatctacacaactgagcacactctttccctacacgac

SEQ ID NO: 93 - DNA, 57 bp, Artificial Sequence
  synthetic nucleic acid
  misc_feature (30)..(37): sample barcode
aatgatacggcgaccaccgagatctacaccttaggacacactctttccctacacgac

SEQ ID NO: 94 - DNA, 57 bp, Artificial Sequence
  synthetic nucleic acid
  misc_feature (30)..(37): sample barcode
aatgatacggcgaccaccgagatctacacgtgccataacactctttccctacacgac

SEQ ID NO: 95 - DNA, 57 bp, Artificial Sequence
  synthetic nucleic acid
  misc_feature (30)..(37): sample barcode
aatgatacggcgaccaccgagatctacacgaatccgaacactctttccctacacgac

SEQ ID NO: 96 - DNA, 57 bp, Artificial Sequence
  synthetic nucleic acid
  misc_feature (30)..(37): sample barcode
aatgatacggcgaccaccgagatctacactcgctgttacactctttccctacacgac

SEQ ID NO: 97 - DNA, 57 bp, Artificial Sequence
  synthetic nucleic acid
  misc_feature (30)..(37): sample barcode
aatgatacggcgaccaccgagatctacacttcgttggacactctttccctacacgac

SEQ ID NO: 98 - DNA, 57 bp, Artificial Sequence
  synthetic nucleic acid
  misc_feature (30)..(37): sample barcode
aatgatacggcgaccaccgagatctacacaagcactgacactctttccctacacgac